European Patent Application EP 4 265 730 A1, published October 25, 2023. Title: Cell-free enzymatic method for preparation of N-glycans. Applicant: Max-Planck-Gesellschaft zur Foerderung der Wissenschaften e.V. The sequence listing filed with the application follows.

SEQUENCE LISTING (37 sequences)

SEQ ID NO: 1 - protein, 10 aa, Artificial Sequence
  synthetic peptide with consensus sequence
GSDANYTYTQ

SEQ ID NO: 2 - protein, 21 aa, Artificial Sequence
  synthetic peptide with consensus sequence
STDTVDTVLEKNVTVTHSVNL

SEQ ID NO: 3 - protein, 713 aa, Artificial Sequence
  Campylobacter jejuni strain RM1221
MLKKEYLKNPYLVLFAMIILAYVFSVLCRFYWIWWASEFNEYFFNNQLMIISNDGYAFAEGARDMIAGFHQPNDLSYYGSSLSTLTYWLYKITPFSFESIILYMSTFLSSLVVIPIILLANEYKRPLMGFVAALLASVANSYYNRTMSGYYDTDMLVIVLPMFILFFMVRMILKKDFFSLIALPLFIGIYLWWYPSSYTLNVALIGLFLIYTLIFHRKEKIFYIAVILSSLTLSNIAWFYQSAIIVILFALFALEQKRLNFMIIGILGSATLIFLILSGGVDPILYQLKFYIFRNDESANLTQGFMYFNVNQTIQEVENVDFSEFMRRISGSEIVFLFSLFGFVWLLRKHKSMIMALPILVLGFLALKGGLRFTIYSVPVMALGFGFLLSEFKAILVKKYSQLTSNVCIVFATILTLAPVFIHIYNYKAPTVFSQNEASLLNQLKNIANREDYVVTWWDYGYPVRYYSDVKTLVDGGKHLGKDNFFPSFALSKDEQAAANMARLSVEYTEKSFYAPQNDILKSDILQAMMKDYNQSNVDLFLASLSKPDFKIDTPKTRDIYLYMPARMSLIFSTVASFSFINLDTGVLDKPFTFSTAYPLDVKNGEIYLSNGVVLSDDFRSFKIGDNVVSVNSIVEINSIKQGEYKITPIDDKAQFYIFYLKDSAIPYAQFILMDKTMFNSAYVQMFFLGNYDKNLFDLVINSRDAKVFKLKI

SEQ ID NO: 4 - protein, 712 aa, Artificial Sequence
  Campylobacter lari strain RM2100 / D67 / ATC BAA-1060
MKLQQNFTDNNSIKYTCILILIAFAFSVLCRLYWVAWASEFYEFFFNDQLMITTNDGYAFAEGARDMIAGFHQPNDLSYFGSSLSTLTYWLYSILPFSFESIILYMSAFFASLIVVPIILIAREYKLTTYGFIAALLGSIANSYYNRTMSGYYDTDMLVLVLPMLILLTFIRLTINKDIFTLLLSPVFIMIYLWWYPSSYSLNFAMIGLFGLYTLVFHRKEKIFYLTIALMIIALSMLAWQYKLALIVLLFAIFAFKEEKINFYMIWALIFISILILHLSGGLDPVLYQLKFYVFKASDVQNLKDAAFMYFNVNETIMEVNTIDPEVFMQRISSSVLVFILSFIGFILLCKDHKSMLLALPMLALGFMALRAGLRFTIYAVPVMALGFGYFLYAFFNFLEKKQIKLSLRNKNILLILIAFFSISPALMHIYYYKSSTVFTSYEASILNDLKNKAQREDYVVAWWDYGYPIRYYSDVKTLIDGGKHLGKDNFFSSFVLSKEQIPAANMARLSVEYTEKSFKENYPDVLKAMVKDYNKTSAKDFLESLNDKDFKFDTNKTRDVYIYMPYRMLRIMPVVAQFANTNPDNGEQEKSLFFSQANAIAQDKTTGSVMLDNGVEIINDFRALKVEGASIPLKAFVDIESITNGKFYYNEIDSKAQIYLLFLREYKSFVILDESLYNSSYIQMFLLNQYDQDLFEQITNDTRAKIYRLKR

SEQ ID NO: 5 - protein, 713 aa, Campylobacter coli
MLKKEYLKNPYLVLFAMIVLAYVFSVFCRFYWVWWASEFNEYFFNNQLMIISNDGYAFAEGARDMIAGFHQPNDLSYYGSSLSTLTYWLYKITPFSFESIILYMSTFLSSLVVIPIILLANEYKRPLMGFVAALLASVANSYYNRTMSGYYDTDMLVIVLPMFILFFMVRMILKKDFFSLIALPLFIGIYLWWYPSSYTLNVALIGLFLIYTLIFHRKEKIFYIAVILSSLTLSNIAWFYQSAIIVILFALFALEQKRLNFMIIGILGSATLIFLILSGGVDPILYQLKFYIFRSDESANLTQGFMYFNVNQTIQEVENVDFSEFMRRISGSEIVFLFSLFGFVWLLRKHKSMIMALPILVLGFLALKGGLRFTIYSVPVMALGFGFLLSEFKAILVKKYSQLTSNVCIVFATILTLAPVFIHIYNYKAPTVFSQNEASLLNQLKNIANREDYVVTWWDYGYPVRYYSDVKTLVDGGKHLGKDNFFPSFSLSKDEQAAANMARLSVEYTEKSFYAPQNDILKSDILQAMMKDYNQSNVDLFLASLSKPDFKIDTPKTRDIYLYMPARMSLIFSTVASFSFINLDTGVLDKPFTFSTAYPLDVKNGEIYLSNGVVLSDDFRSFKIGDNVVSVNSIVEINSIKQGEYKITPIDDKAQFYIFYLKDSAIPYAQFILMDKTMFNSAYVQMFFLGNYDKNLFDLVINSRDAKVFKLKI

SEQ ID NO: 6 - protein, 785 aa, Campylobacter upsaliensis
MKNEAVKNANLRLVFFILLAFGFSVLCRFYWIYWASDFNEYFFNNQLMISSNDGYTFAEGARDKIAGFHQENDLSFINSSLSILTYVLYKITPFSFESIILYMSVFFSSLIVVPLILIANELKRPLMGLFAAFLASIAKSYYNRTMAGYYDTDMLAIVLPMFILYFFIRLVLRKDDFSLLALPFFMGLYLWWYPSSYTLNVAFIALFTLYVLIYHRKERSFYMAALLCAITLSNIAWFYQSAIVVLFFAFFMLKNSLFNFKFIALLALGVLVFLVLSGGIDPILYQLKFYLLRSDESASLARGFAYFNVNLTIQEVESIDLSTFMQRISGSELVFLLSLFGFLWLLKKHKIMLLTLPMLLLGFLALRGGLRFTIYAVPIMALGFGFLSVQLLSLIQKMRPLQETRKLRIFFYGIFPLFVLVLGAYFYFSQSAIYESMGVEFQKSFVSFFVEDTLLFSLLVLALFTPLIFELLWRKKDIRFVCSFYIVGVLLFSLWANLSHIYNYRAHTVFNYNEASILDNLKANVSREDYIVAWWDYGYPIRYYSDVKTLADGGKHLGKDNFFPSFVLSQNPRAAANMARLSVEYTEKSFKTPYNDLLEAMMKDYNFNNVNLFLAALSKEDFTIQTPKTRDIYIYMPSRMAAIFGTVASFSYMSLETGELENPFVYSVAYYLGNEDGKLVLSNNMLLHSDFRSFELNGKNYAINSLVEFTSVQQKYYSVVEIDKNAKYYLFHIKDANIPNVQFILMDKAMYESAFVQMFFFGKYDESLYELIVDSKEAKVYKLKL

SEQ ID NO: 7 - protein, 816 aa, Desulfovibrio desulfuricans strain DSM 7057
MPHQSLENSSSEQAANHPACNAGGGCNDAVAHTAEHSCATSTAHSVALRERGHPLALPRAVHLGLPPGPDVAGYWLRGFFWGVVTLVLAFGLRMLEWPCWQDPEFRLGSQWLLATHDAYHWVAGAEGIGLAVGHPMAEMLRWMADALGTYPAAVAFWFPAVLASFVALIVYAWVWALGSMEAGVAAGLLTSLAPGFLARTLLGYYDTDLVTLFFPLLMTLAPASWAMRYMLLPQMVLRRMAIGAGIMTARRLFSRGLPEDKLVRQLGQGEHLGNPLRWQWVVLLGCSGVISWWTQEWHSVFPYLIRYNVILLAFMSLIMAPRGRRALLLLGSLAYALPTLTGPVGLVFSLLLLLAGTRPGLKARRVLCRPGVLSLLWVGVAFLLVQGEILTTLTNHVNAYLKHAGDAKSTGEGAVLMYPSVAQSIIEVQDLSFAALFPYFHPWMEASIVGLLGFVVVMVRRPGALFLLPLAALGLLSTKLGGRMVMFGAPVVAVGLTLPLFWTWQRLLRTSLRGSVAGLLTSAVLIALMVAPFVDMIPAMSQGPMINRRHAEALTRARTMTPEDSMLWLWWDWGYAAHYFAHRATIADGAQHAGPSLYLPAAVFATDNARFARQLIRYTAQRGNEPGNVFEGLDGTSAQVLMDRLRSDETPLIEARGRLFVVVSFEMLRLGFWISNFGNWNFITHSGEGGALSIVPQELAYRLDSGEVRLEGSTSAIYASSINVFEETGVTRRNYVQEWFDAHPDASPQEQQDFLSRRRNVNFLFNRITDEKLAMDEGLYNSLMVQLLVGDPQSPRFSPYFKLVYDNVFARIYEVL

SEQ ID NO: 8 - protein, 715 aa, Megalodesulfovibrio gigas DSM 1382
MSAPWNAVAPEQPARQELKLFLFVLGFTYALALAVHMHEIYGWQNPALVVDGEFIQGTHDSYHWLAGAKGVGEAVGTPLAVMAAGFASLTGMPLGLAGFVIPPLFAGLVGLVMAVWCRVLGWKEGAAAGGLVAGLLTVLSPGFYFRSRLGYYDTDMVTLLFPLLFTLGLAMAMGRWIRPSWRHREPLQEEPPQTIARVLAWLVLLGLLARFGAVWHGHILTFVKVLCGFSVCWGLAAGRPGARGRLMLGLAVFMASALVGWPGLACSLALWALAWKKPEMVSQWARAPWPGLAALVLLAVLGGVAQTTLQSATELLGAYLKPAADVTGSVNTTGVIYPGIGQSVIEVQNIALERVLERFHTSWLVAATGLLCFLGVLVLRPVALPLAIFLVMGLASVKLGSRLTMFGGAPMAIGLGMAVGWAGVALFRSGPGAGYKRFLLSCAATVVLGWPLVSFYISLPPTPVLSRQHCMALQSLKTSPPESKVWTWWDWGYPTHYYAERISFADGGRHYGHHIFPLGLVLTTPNPRLSAQLIKYSAQWNDEPWKAWDAMPRNEMLALLQGLGNATQPLPPFAAPRYVVATFENIRLAPWITYYGTWDMTTQQGLHGRLLEIRDAFRINYEKGEVQFTQREGVLPVASIDVLDRKERRSDVFPRNQGPHLVVHMAAQKYYLLDDQIYNSMMVQLLLEDPKKPRFGDYFSLVYDDFPDVRVFEVR

SEQ ID NO: 9 - protein, 758 aa, Desulfovibrio vulgaris
MTRLRGTLSVCIDAFPAWTRPLALAFVVYALSFGMRMLEYPAWQNPEYMLDGEYLLATHDAYHWIAGAEGFEFGAGHPMSELVRLAAAFTGTTPAAVGFWLPPVMASLVAVGVFGWAAALGGVEAGVCAGVLASLAPGFLARTLLGYCDTDLVTLLFPLLMGLGPAFWMARFMFTPLQVARRLLARRTGTSDVVPDAVAVMMTSRGEADDDWHGGALSPRWLALLAGSGLVGSWGAEWHSLFPYLIRYDVVLLFGCICVFGRPGMRRALLVGGLAYALPMLVGAWGLLFALALGWGLHRADARFMAFVRGRALPVAGWCAVAVLLFDPDVFRMFLNSIAGYVKRSGDPSPGAGGDDPLVYPSVAQSIIEVQDLSLSEVLSYFHPWLWVALAGLGGFVPLLLARPAAFFLLPLGVLSFLSVKLGGRMVMFGAPVLALGFALPMVWGVQRVLRHDLRTGWVRLALSAVLLVIVATPFVDLLPAMTQGPIINKRHAEALRHIRTATPEDSMVWIWWDWGYSAHHFAHRRTIADGASHGGPSLYVPAAVFSTANPRFAWQLIRYTAERGGIPGSVFEGMGGAQAQELVHRLGIEKMTFADAPRQYLVVSYDMLRLGFWITNFGTWDFLSREGKGYAISSIPQQLSYSLDTGEVQVQGNTTGVLASTIDVFDEGQLERRDYIVRQGGSGNAIADYAARQRNIESRRNIHFLFNKVTGEKLVLDDRLYNTVMVQLLLCSPDDTRFAPYFKLIYDNVYARVYEVR

SEQ ID NO: 10 - protein, 827 aa, Trypanosoma brucei
MTKGGKVAVTKGSAQSDGAGEGGMSKAKSSTTFVATGGGSLPAWALKAVSTIVSAVILIYSVHRAYDIRLTSVRLYGELIHEFDPWFNYRATQYLSDNGWRAFFQWYDYMSWYPLGRPVGTTIFPGMQLTGVAIHRVLEMLGRGMSFPGMQLTGVAIHRVLEMLGRGMSINNICVYIPAWFGSIATVLAALIAYESSNSLSVMAFTAYFFSIVPAHLMRSMAGEFDNECVAMAAMLLTFYMWVRSLRSSSSWPIGALAGVAYGYMVSTWGYIFVLNMVAFHASVCVLLDWARGTYSVSLLRAYSLFFVIGTALAICVPPVEWTPFRSLEQLTALFVFVFMWALHYSEYLRERARAPIHSSKALQIRARIFMGTLSLLLIVASLLAPFGFFKPTAYRVRALFVKHTRTGNPLVDSVAEHRPTTAGAYLRYFHVCYPLWGCGGLSMLVFMKKDRWRAIVFLASLSTVTMYFSARMSRLLLLAGPAATACAGMFIGGLFDLALSQFGDLRSPKDASGDSDPAGGSKRAKGKVVNEPSERAIFSHRWFQRLVQSLPVPLRRGIAVVVLVCLFANPMRHSFEKSCEKMAHALSSPRIIAVTDLPNGERVLADDYYVSYLWLRNNTPEDARILSWWDYGYQITGIGNRTTLADGNTWSHKHIATIGKMLTSPVKESHALIRHLADYVLIWAGYDGSDLLKSPHMARIGNSVYRDMCSEDDPLCRQFGFYSGDLNKPTPMMQRSLLYNLHRFGTDGGKTQLDKNMFQLAYVSKYGLVKIYKVMNVSEESKAWVADPKNRVCDPPGSWICAGQYPPAKEIQDMLAKRFHYEASSR

SEQ ID NO: 11 - protein, 718 aa, Saccharomyces cerevisiae strain ATCC 204508 / S288c
MGSDRSCVLSVFQTILKLVIFVAIFGAAISSRLFAVIKFESIIHEFDPWFNYRATKYLVNNSFYKFLNWFDDRTWYPLGRVTGGTLYPGLMTTSAFIWHALRNWLGLPIDIRNVCVLFAPLFSGVTAWATYEFTKEIKDASAGLLAAGFIAIVPGYISRSVAGSYDNEAIAITLLMVTFMFWIKAQKTGSIMHATCAALFYFYMVSAWGGYVFITNLIPLHVFLLILMGRYSSKLYSAYTTWYAIGTVASMQIPFVGFLPIRSNDHMAALGVFGLIQIVAFGDFVKGQISTAKFKVIMMVSLFLILVLGVVGLSALTYMGLIAPWTGRFYSLWDTNYAKIHIPIIASVSEHQPVSWPAFFFDTHFLIWLFPAGVFLLFLDLKDEHVFVIAYSVLCSYFAGVMVRLMLTLTPVICVSAAVALSKIFDIYLDFKTSDRKYAIKPAALLAKLIVSGSFIFYLYLFVFHSTWVTRTAYSSPSVVLPSQTPDGKLALIDDFREAYYWLRMNSDEDSKVAAWWDYGYQIGGMADRTTLVDNNTWNNTHIAIVGKAMASPEEKSYEILKEHDVDYVLVIFGGLIGFGGDDINKFLWMIRISEGIWPEEIKERDFYTAEGEYRVDARASETMRNSLLYKMSYKDFPQLFNGGQATDRVRQQMITPLDVPPLDYFDEVFTSENWMVRIYQLKKDDAQGRTLRDVGELTRSSTKTRRSIKRPELGLRV

SEQ ID NO: 12 - protein, 826 aa, Homo sapiens
MAEPSAPESKHKSSLNSSPWSGLMALGNSRHGHHGPGAQCAHKAAGGAAPPKPAPAGLSGGLSQPAGWQSLLSFTILFLAWLAGFSSRLFAVIRFESIIHEFDPWFNYRSTHHLASHGFYEFLNWFDERAWYPLGRIVGGTVYPGLMITAGLIHWILNTLNITVHIRDVCVFLAPTFSGLTSISTFLLTRELWNQGAGLLAACFIAIVPGYISRSVAGSFDNEGIAIFALQFTYYLWVKSVKTGSVFWTMCCCLSYFYMVSAWGGYVFIINLIPLHVFVLLLMQRYSKRVYIAYSTFYIVGLILSMQIPFVGFQPIRTSEHMAAAGVFALLQAYAFLQYLRDRLTKQEFQTLFFLGVSLAAGAVFLSVIYLTYTGYIAPWSGRFYSLWDTGYAKIHIPIIASVSEHQPTTWVSFFFDLHILVCTFPAGLWFCIKNINDERVFVALYAISAVYFAGVMVRLMLTLTPVVCMLSAIAFSNVFEHYLGDDMKRENPPVEDSSDEDDKRNQGNLYDKAGKVRKHATEQEKTEEGLGPNIKSIVTMLMLMLLMMFAVHCTWVTSNAYSSPSVVLASYNHDGTRNILDDFREAYFWLRQNTDEHARVMSWWDYGYQIAGMANRTTLVDNNTWNNSHIALVGKAMSSNETAAYKIMRTLDVDYVLVIFGGVIGYSGDDINKFLWMVRIAEGEHPKDIRESDYFTPQGEFRVDKAGSPTLLNCLMYKMSYYRFGEMQLDFRTPPGFDRTRNAEIGNKDIKFKHLEEAFTSEHWLVRIYKVKAPDNRETLDHKPRVTNIFPKQKYLSKKTTKRKRGYIKNKLVFKKGKKISKKTV

SEQ ID NO: 13 - protein, 823 aa, Mus musculus
MAEPSAPESKHKSSLNSSPWSGLMALGNSRHGHHGPGTQSASSAAAPKPGPPAGLSGGLSQPAGWQSLLSFTILFLAWLAGFSSRLFAVIRFESIIHEFDPWFNYRSTHHLASHGFYEFLNWFDERAWYPLGRIVGGTVYPGLMITAGLIHWILNTLNITVHIRDVCVFLAPTFSGLTSISTFLLTRELWNQGAGLLAACFIAIVPGYISRSVAGSFDNEGIAIFALQFTYYLWVKSVKTGSVFWTMCCCLSYFYMVSAWGGYVFIINLIPLHVFVLLLMQRYSKRVYIAYSTFYIVGLILSMQIPFVGFQPIRTSEHMAAAGVFALLQAYAFLQYLRDRLTKQEFQTLFFLGVSLAAGAVFLSVIYLTYTGYIAPWSGRFYSLWDTGYAKIHIPIIASVSEHQPTTWVSFFFDLHILVCTFPAGLWFCIKNINDERVFVALYAISAVYFAGVMVRLMLTLTPVVCMLSAIAFSNVFEHYLGDDMKRENPPVEDSSDEDDKRNPGNLYDKAGKVRKHVTEQEKPEEGLGPNIKSIVTMLMLMLLMMFAVHCTWVTSNAYSSPSVVLASYNHDGTRNILDDFREAYFWLRQNTDEHARVMSWWDYGYQIAGMANRTTLVDNNTWNNSHIALVGKAMSSNETAAYKIMRSLDVDYVLVIFGGVIGYSGDDINKFLWMVRIAEGEHPKDIREGDYFTQQGEFRVDKAGSPTLLNCLMYKMSYYRFGEMQLDFRTPPGFDRTRNAEIGNKDIKFKHLEEAFTSEHWLVRIYKVKAPDNRETLGHKPRVTNIVPKQKYLSKKTTKRKRGYVKNKLVFKKGKKTSKKTV

SEQ ID NO: 14 - protein, 752 aa, Schizosaccharomyces pombe strain 972 / ATCC 24843
MANSATITSKKGVKSHQKDWKIPLKVLILICIAVASVSSRLFSVIRYESIIHEFDPWFNFRASKILVEQGFYNFLNWFDERSWYPLGRVAGGTLYPGLMVTSGIIFKVLHLLRINVNIRDVCVLLAPAFSGITAIATYYLARELKSDACGLLAAAFMGIAPGYTSRSVAGSYDNEAIAITLLMSTFALWIKAVKSGSSFWGACTGLLYFYMVTAWGGYVFITNMIPLHVFVLLLMGRYTSKLYIAYTTYYVIGTLASMQVPFVGFQPVSTSEHMSALGVFGLLQLFAFYNYVKGLVSSKQFQILIRFALVCLVGLATVVLFALSSTGVIAPWTGRFYSLWDTNYAKIHIPIIASVSEHQPPTWSSLFFDLQFLIWLLPVGVYLCFKELRNEHVFIIIYSVLGTYFCGVMVRLVLTLTPCVCIAAAVAISTLLDTYMGPEVEEDKVSEEAASAKSKNKKGIFSILSFFTSGSKNIGIYSLLSRVLVISSTAYFLIMFVYHSSWVTSNAYSSPTVVLSTVLNDGSLMYIDDFREAYDWLRRNTPYDTKVMSWWDYGYQIAGMADRITLVDNNTWNNTHIATVGKAMSSPEEKAYPILRKHDVDYILIIYGGTLGYSSDDMNKFLWMIRISQGLWPDEIVERNFFTPNGEYRTDDAATPTMRESLLYKMSYHGAWKLFPPNQGYDRARNQKLPSKDPQLFTIEEAFTTVHHLVRLYKVKKPDTLGRDLKQVTLFEEGKRKKLRRPAKTNEIPLRV

SEQ ID NO: 15 - protein, 826 aa, Canis lupus familiaris
MAEPSAPESKHKSSLNSSPWSGLMALGNSRHGHHGPGAQCAHKAAGGVAPPKPAPAGLSGGLSQPAGWQSLLSFTILFLAWLAGFSSRLFAVIRFESIIHEFDPWFNYRSTHHLASHGFYEFLNWFDERAWYPLGRIVGGTVYPGLMITAGLIHWILNTLNITVHIRDVCVFLAPTFSGLTSISTFLLTRELWNQGAGLLAACFIAIVPGYISRSVAGSFDNEGIAIFALQFTYYLWVKSVKTGSVFWTMCCCLSYFYMVSAWGGYVFIINLIPLHVFVLLLMQRYSKRVYIAYSTFYIVGLILSMQIPFVGFQPIRTSEHMAAAGVFALLQAYAFLQYLRDRLTKQEFQTLFFLGVSLAAGAVFLSVIYLTYTGYIAPWSGRFYSLWDTGYAKIHIPIIASVSEHQPTTWVSFFFDLHILVCTFPAGLWFCIKNINDERVFVALYAISAVYFAGVMVRLMLTLTPVVCMLSAIAFSNVFEHYLGDDMKRENPPVEDSSDEDDKRNPGNLYDKAGKVRKHVTEQEKTEEGLGPNIKSIVTMLMLMLLMMFAVHCTWVTSNAYSSPSVVLASYNHDGTRNILDDFREAYFWLRQNTDEHARVMSWWDYGYQIAGMANRTTLVDNNTWNNSHIALVGKAMSSNESAAYKIMRSLDVDYVLVIFGGVIGYSGDDINKFLWMVRIAEGEHPKDIRESDYFTPQGEFRVDKAGSPTLLNCLMYKMSYYRFGEMQLDFRTPPGFDRTRNAEIGNKDIKFKHLEEAFTSEHWLVRIYKVKAPDNRETLDHKPRVTNIFPKQKYLSKKTTKRKRGYIKNKLVFKKGKKISKKTV

SEQ ID NO: 16 - protein, 779 aa, Arabidopsis thaliana
MAALESPLPGTPTAMRNAFGNVLSVLILVLIGVLAFSIRLFSVIKYESVIHEFDPYFNYRVTQFLSKNGIYEFWNWFDDRTWYPLGRVIGGTVYPGLTLTAGTIWWGLNSLNIPLSVETVCVFTAPVFSAFASWATYLLTKEVKGSGAGLAAAALLAMVPSYISRSVAGSYDNEAVAIFALIFTFYLYIKTLNTGSLFYATLNALAYFYMVCSWGGYTFIINLIPMHVLLCIVTGRYSPRLYIAYAPLVVLGTLLAALVPVVGFNAVLTSEHFASFLVFIIIHVVALVYYIKGILSPKMFKVAVTLVVSIGMVVCFIVVAILVALVASSPTGGWSGRSLSLLDPTYASKYIPIIASVSEHQPPTWPSYFMDINVLAFLVPAGIIACFSPLSDASSFVVLYIVMSVYFSGVMVRLMLVLAPAACIMSGIALSQAFDVFTGSIKYQLGASSNSTDDAEDNTSTNNAPKDDVSAGKTDKGEEIVKERSSKKGKKKEREPADKPSVKAKIKKKALVLPLEASIVALLLLIMLGAFYVIHCVWAAAEAYSAPSIVLTSQSRDGLHVFDDFRESYAWLSHNTDVDDKVASWWDYGYQTTAMANRTVIVDNNTWNNTHIATVGTAMSSPEKAAWEIFNSLDVKYVLVVFGGLIGYPSDDINKFLWMVRIGGGVFPHIKEADYLRDGQYRIDSEATPTMLNSLMYKLSYYRFVETDGKGYDRVRRTEIGKKHFKLTHFEEVFTSHHWMVRLYKLKPPRNRIRGKAKKLKSKTSSGLSSKSAKKNPWV

SEQ ID NO: 17 - protein, 705 aa, Canis lupus familiaris
MTKLGFLRLSYEKQDTLLKLLILSMAAVLSFSTRLFAVLRFESVIHEFDPYFNYRTTRFLAEEGFYKFHNWFDDRAWYPLGRIIGGTIYPGLMITSAAIYHVLHFFHITIDIRNVCVFLAPLFSSFTTIVTYHLTKELKDAGAGLLAAAMIAVVPGYISRSVAGSYDNEGIAIFCMLLTYYMWIKAVKTGSIYWAAKCALAYFYMVSSWGGYVFLINLIPLHVLVLMLTGRFSHRIYVAYCTVYCLGTILSMQISFVGFQPVLSSEHMAAFGVFGLCQIHAFVDYLRSKLNPQQFEVLFRSVISLVGFVLLTVGALLMLTGKISPWTGRFYSLLDPSYAKNNIPIIASVSEHQPTTWSSYYFDLQLLVFMFPVGLYYCFSNLSDARIFIIMYGVTSMYFSAVMVRLMLVLAPVMCILSGIGVSQVLSTYMKNLDISRPDKKSKKQQDSTYPIKNEVASGMILVMAFFLITYTFHSTWVTSEAYSSPSIVLSARGGDGSRIIFDDFREAYYWLRHNTPEDAKVMSWWDYGYQITAMANRTILVDNNTWNNTHISRVGQAMASTEEKAYEIMRELDVSYVLVIFGGLTGYSSDDINKFLWMVRIGGSTDTGKHIKEHDYYTPTGEFRVDREGSPVLLNCLMYKMCYYRFGQVYTEAKRPPGFDRVRNAEIGNKDFELDVLEEAYTTEHWLVRIYKVKDLDNRGLSRT

SEQ ID NO: 18 - protein, 735 aa, Arabidopsis thaliana
MGGKSEPAKSESMATKPDLLNTSFFSFKSLKLKTKQQELLLRISILGLVYILAFIARLFSVLRYESMIHEFDPYFNYRTTLFLTEKGFYEFWNWFDSESWYPLGRIIGGTLYPGLMVTAALIYWTLRFLRFFVHIREVCVLTAPFFASNTTLVAYFFGKELWDTGAGLVAAVLIAICPGYISRSVAGSYDNEAVAIFALLLTFYLFVKAVNTGSLAWALASAFGYFYMVSAWGGYVFIINLVPLYVLVLLITGRYSMRLYIAYNCMYILGMLLAMQIRFVGFQHVQSGEHMGAMGVFLLMQVFYFLDWVKYQLNDTKLFQTFLRITVTSAILVGGVAVGVGTASGYISPWTGRFYSLLDPTYAKDHIPIIASVSEHQPTAWSSFMFDYHILLFLFPAGLYFCFKRLTDATIFIVMYGLTSLYFAGVMVRLILVATPAVCLISAIAVSATIKNLTSLLRTKQKVSQTGSTKGAGSSKASSKVTLDQSQPFQKNGAIALLVGVFYLLSRYAIHCTWVTAEAYSSPSIVLAARGAHGNRIIFDDYREAYYWLRQNTATDAKIMSWWDYGYQITAMGNRTVIVDNNTWNNTHIATVGRAMSSYEDDAYDIMRSLDVNYVLVVFGGVTGYSSDDINKFLWMVRIGGGVFPVIKEPDYLVNGEFRVDKGASPKMLNCLMYKLCYYRFGELTTEYGKPPGYDRARGVEIGNKDIKLEHLEEAYTTSNWIVRIYRVKPPTNRL

SEQ ID NO: 19 - protein, 757 aa, Caenorhabditis elegans
MTSTTAARTASSRVGATTLLTIVVLALAWFVGFASRLFAIVRFESIIHEFDPWFNYRATHHMVQHGFYKFLNWFDERAWYPLGRIVGGTVYPGLMVTSGLIHWILDSLNFHVHIREVCVFLAPTFSGLTAIATYLLTKELWSPGAGLFAACFIAISPGYTSRSVAGSYDNEGIAIFALQFTYYLWVKSLKTGSIMWASLCALSYFYMVSAWGGYVFIINLIPLHALALIIMGRYSSRLFVSYTSFYCLATILSMQVPFVGFQPVRTSEHMPAFGVFGLLQIVALMHYARNRITRQQFMTLFVGGLTILGALSVVVYFALVWGGYVAPFSGRFYSLWDTGYAKIHIPIIASVSEHQPTTWVSFFFDLHITAAVFPVGLWYCIKKVNDERVFIILYAVSAVYFAGVMVRLMLTLTPAVCVLAGIGFSYTFEKYLKDEETKERSSSQSGTTKDEKLYDKAAKNVKSRNANDGDESGVSSNVRTIISIILVIFLLMFVVHATYVTSNAYSHPSVVLQSSTNNGDRIIMDDFREAYHWLRENTADDARVMSWWDYGYQIAGMANRTTLVDNNTWNNSHIALVGKAMSSNESAAYEIMTELDVDYILVIFGGVIGYSGDDINKFLWMVRIAQGEHPKDIREENYFTSTGEYSTGAGASETMLNCLMYKMSYYRFGETRVGYNQAGGFDRTRGYVIGKKDITLEYIEEAYTTENWLVRIYKRKKLPNRPTVKSEEATIPIKGKKATQGKNKKGVIRPAPTASKA

SEQ ID NO: 20 - protein, 705 aa, Bos taurus
MTKLGFLRLSYEKQDTLLKLLILSMAAVLSFSTRLFAVLRFESVIHEFDPYFNYRTTRFLAEEGFYKFHNWFDDRAWYPLGRIIGGTIYPGLMITSAAIYHVLHFFHITIDIRNVCVFLAPLFSSFTTIVTYHLTKELKDAGAGLLAAAMIAVVPGYISRSVAGSYDNEGIAIFCMLLTYYMWIKAVKTGSIYWAAKCALAYFYMVSSWGGYVFLINLIPLHVLVLMLTGRFSHRIYVAYCTVYCLGTILSMQISFVGFQPVLSSEHMAAFGVFGLCQIHAFVDYLRSKLNPQQFEVLFRSVISLVGFVLLTIGALLMLTGKISPWTGRFYSLLDPSYAKNNIPIIASVSEHQPTTWSSYYFDLQLLVFMFPVGLYYCFSNLSDARIFIIMYGVTSMYFSAVMVRLMLVLAPVMCILSGIGVSQVLSTYMKNLDISRQDKKSKKQQDSTYPIKNEVASGMILVMAFFLITYTFHSTWVTSEAYSSPSIVLSARGGDGSRIIFDDFREAYYWLRHNTPEDAKVMSWWDYGYQITAMANRTILVDNNTWNNTHISRVGQAMASTEEKAYEIMRELDVSYVLVIFGGLTGYSSDDINKFLWMVRIGGSTDTGKHIKEHDYYTPTGEFRVDREGSPVLLNCLMYKMCYYRFGQVYTEAKRPLGYDRVRNAEIGNKDFELDVLEEAYTTEHWLVRIYKVKDLDNRGLSRT

SEQ ID NO: 21 - protein, 705 aa, Pongo pygmaeus abelii
MTKFGFLRLSYEKQDTLLKLLILSMAAVLSFSTRLFAVLRFESVIHEFDPYFNYRTTRFLAEEGFYKFHNWFDDRAWYPLGRIIGGTIYPGLMITSAAIYHVLHFFHITIDIRNVCVFLAPLFSSFTTIVTYHLTKELKDAGAGLLAAAMIAVVPGYISRSVAGSYDNEGIAIFCMLLTYYMWIKAVKTGSICWAAKCALAYFYMVSSWGGYVFLINLIPLHVLVLMLTGRFSHRIYVAYCTVYCLGTILSMQISFVGFQPVLSSEHMAAFGVFGLCQIHAFVDYLRSKLNPQQFEVLFRSVISLVGFVLLTVGALLMLTGKISPWTGRFYSLLDPSYAKNNIPIIASVSEHQPTTWSSYYFDLQLLVFMFPVGLYYCFSNLSDARIFIIMYGVTSMYFSAVMVRLMLVLAPVMCILSGIGVSQVLSTYMKNLDISRPDKKSKKQQDSTYPIKNEVASGMILVMAFFLITYTFHSTWVTSEAYSSPSIVLSARGGDGSRIIFDDFREAYYWLRHNTPEDAKVMSWWDYGYQITAMANRTILVDNNTWNNTHISRVGQAMASTEEKAYEIMRELDVSYVLVIFGGLTGYSSDDINKFLWMVRIGGSTDTGKHIKENDYYTPTGEFRVDREGSPVLLNCLMYKMCYYRFGQVYTEAKRPPGFDRVRNAEIGNKDFELDVLEEAYTTEHWLVRIYKVKDLDNRGLSRT

SEQ ID NO: 22 - protein, 787 aa, Oryza stiva japonica
MAEPESSTAAAGGSRLRNACGGVLCAFTLLLIGVLAFSIRLFSVIKYESVIHEFDPYFNFRVTQFLSKNGIYEFWNWFDDRTWYPLGRVIGGTVYPGLTLTAGTIWWLLNSLNIPLSVETVCVFTAPIFSANASWATYLLTKEAKGTGAGLMAAAILAMVPSYISRSVAGSYDNEAVAIFALIFTFYLYVKTLNTGSLFYATLNALSYFYMVCSWGGYTFIINLIPIHVLLCIVTGRYSSRLYIAYAPLVILGTLLAALVPVVGFNAVMTSEHFASFLVFIILHVVALVYYIKGLLTPRLFKVAMTLVITVGLAVCFAVIAILIALVASSPTKGWSGRSLSLLDPTYASKYIPIIASVSEHQPPTWPSYFMDINVLAFLIPAGIISCFLPLSDASSFVVLYLVTAVYFSGVMVRLMLVLAPAACILSGIALSEAFDVLTRSVKYQLSKLFDDSPAASGDSSAESSSASTVSTNSAKNETRPEKTETAPKEKPSKKNRKKEKEVAESVPVKPKKEKKLLVLPMEASVLGILLLIVLGGFYVVHCVWAAAEAYSAPSIVLTSRSRDGLHVFDDFREAYAWLSHNTDVDDKVASWWDYGYQTTAMANRTVIVDNNTWNNTHIATVGTAMSSPEKAAWEIFNSLDVKYVLVVFGGLVGYPSDDINKFLWMVRIGGGVFPHIKEPDYLRDGNYRVDAQGTPTMLNCLMYKLCYYRFVETDGKGFDRVRGYEIGKKHFKLTHFEEVFTTHHWMVRIYKLKPQKNRVRGKLKKLKSGSKASSTNAAGRKKNPWQ

SEQ ID NO: 23 - protein, 721 aa, Oryza stiva japonica
MAAATALDSLPAPLRSLRLKTKQQELLLRVSALALIYVLAFVVRLFSVLRYESMIHEFDPYFNYRTTLFLSDHGFSEFWNWFDFESWYPLGRVVGGTLFPGLMVTAALLHRLLRALSLAVHIREVCVLTAPFFAANTTLVAYAFGREIWDSGAGLVAAALIAVCPGYISRSVAGSYDNEGVAIFALLLTFYLFVRAVNTGSLAWSLASAFGYFYMVSAWGGYVFIINLLPLYVLVLLVTGRYSQRLYVAYNSTYVLGMLLAMQIRFVGFQHVQSGEHMAAMGVFFLLQVFFFLDWVKYLLNDAKLFKSFLRITLTCVITVGTLALGIGTASGYISPWTGRFYSLLDPTYAKDHIPIIASVSEHQPTAWSSFMFDFHILLFLFPAGLYFCFKRLSDATIFIVMYGLTSMYFAGVMVRLILVAAPAVCLISAIAASATIKNLTTLIRTKSKSPQTVSGKSSGSKAAAKGAVDQSLPFQQNVAIALLLGAFYLLSRYAVHCTWVTSEAYSSPSIVLAARGHNGGRVIFDDYREAYYWLRQNTPSDAKIMSWWDYGYQITAMGNRTVIVDNNTWNNTHIATVGRAMSSYEDEAYEIMQSLDVNYVLVVFGGVTGYSSDDINKFLWMVRIGGGVFPVIKEPDYLVNGEYRVDKGAAPKMLNCLMYKLCYYRFGELTTEYGKPPGYDRVRGVEIGNKDIKLEYLEEAFTTSNWIVRIYKVKPPKNRS

SEQ ID NO: 24 - protein, 714 aa, Dictyostelium discoideum
MKRSEKSSTSVVSNNKQQDVNIISSNEVGVKEENKGHQEFLLKVLILSVIYVLAFSTRLFSVLRYESVIHEFDPYFNYRSTIYLVQEGFYNFLNWFDERAWYPLGRIVGGTIYPGLMATASLVHWSLNSLNITVNIRNVCVLLSPWFASNTAMVTYKFAKEVKDTQTGLVAAAMIAIVPGYISRSVAGSFDNEGIAIFALIFTYYCWIKSVNTGSLMWAAICSLAYFYMASAWGGYVFIINLIPLHAFFLLLTGRYSHRLYIAYSTMFVIGTILSMQITFISFQPVQSSEHLAAIGIFGLLQLYAGLSWVKSHLTNEAFKKLQRLTVLFVLSCAAAVLVVGTLTGYISPFNGRFYSLLDPTYARDHIPIIASVSEHQPTTWASYFFDLHILVFLFPAGLYFCFQKLTDANIFLILYGVTSIYFSGVMVRLMLVLAPVACILAAVAVSATLTTYMKKLKAPSSPSDANNSKESGGVMVAVLTVLLILYAFHCTWVTSEAYSSPSIVLSAKQNDGSRVIFDDFREAYRWIGQNTADDARIMSWWDYGYQLSAMANRTVLVDNNTWNNSHIAQVGKAFASTEEDAYIQMKALDVDYVLVIFGGLTGYSSDDINKFLWMVRIGGSCDPNIKEQDYLTNGQYRIDKGASPTMLNSLMYKLSYYRFSEVHTDYQRPTGFDRVRNVEIGNKNFDLTYLEEAFTSVHWLVRVYKVKDFDNRA

SEQ ID NO: 25 - protein, 111 aa, Brachypodium distachyon
LSHNTEVEDKVASWWDYGYQTTAMANRTVIVDNNTWNNTHIATVGTAMSSPEKAAWEIFNSLDVKYVLVVFGGLIGYPSDDINKFLWMVRIGGGVFPHIKEQDYLKDGNYR

SEQ ID NO: 26 - protein, 111 aa, Brachypodium retusum
LSHNTDVDDKVASWWDYGYQTTAMANRTVIVDNNTWNNTHIATVGTAMSSPEKAAWEIFDSLDVKYVLVVFGGLVGYPSDDINKFLWMVRIGGGEFPHIKEPDYLRDGQYR

SEQ ID NO: 27 - protein, 824 aa, Rattus norvegicus
MAEPSAPESKHKSSLNSSPWSGLMALGNSRHGHHGPGAQSASRAAAAPKPGPPAGLSGGLSQPAGWQSLLSFTILFLAWLAGFSSRLFAVIRFESIIHEFDPWFNYRSTHHLASHGFYEFLNWFDERAWYPLGRIVGGTVYPGLMITAGLIHWILNTLNITVHIRDVCVFLAPTFSGLTSISTFLLTRELWNQGAGLLAACFIAIVPGYISRSVAGSFDNEGIAIFALQFTYYLWVKSVKTGSVFWTMCCCLSYFYMVSAWGGYVFIINLIPLHVFVLLLMQRYSKRVYIAYSTFYIVGLILSMQIPFVGFQPIRTSEHMAAAGVFALLQAYAFLQYLRDRLTKQEFQTLFFLGVSLAAGAVFLSVIYLTYTGYIAPWSGRFYSLWDTGYAKIHIPIIASVSEHQPTTWVSFFFDLHILVCTFPAGLWFCIKNINDERVFVALYAISAVYFAGVMVRLMLTLTPVVCMLSAIAFSSVFEHYLGDDMKRENPPVEDSSDEDDRRSPGNLYDKAGKVRKHVTEQEKPEEGLGPNIKSIVTMLMLMLLMMFAVHCTWVTSNAYSSPSVVLASYNHDGTRNILDDFREAYFWLRQNTDEHARVMSWWDYGYQIAGMANRTTLVDNNTWNNSHIALVGKAMSSNETAAYKIMRSLDVDYVLVIFGGVIGYSGDDINKFLWMVRIAEGEHPKDIREGDYFTQQGEFRVDRAGSPTLLNCLMYKMSYYRFGEMQLDFRTPPGFDRTRNAEIGNKDIKFKHLEEAFTSEHWLVRIYKVKAPDNRETLGHKPRVTNIFPKQKYLSKKTTKRKRGYVKNKLVFKKGKKMSKKTV

SEQ ID NO: 28 - protein, 109 aa, Brachypodium sylvaticum
HNTDVDDKVASWWDYGYQTTAMANRTVIVDNNTWNNTHIATVGTAMSSPEKAAWEIFDSLDVKYVLVVFGGLVGYPSDDINKFLWMVRIGGGEFPHIKEPDYLRDGQYR

SEQ ID NO: 29 - protein, 111 aa, Brachypodium pinnatum
LSHNTEVEDKVASWWDYGYQTTAMANRTVIVDNNTWNNTHIATVGIAMSSPEKAAWEIFNSLDVKYVLVVFGGLIGYPSDDINKFLWMVRIGGGVFPHIKEQDYLKDGNYR

SEQ ID NO: 30 - protein, 111 aa, Brachypodium rupestre; identical to SEQ ID NO: 25

SEQ ID NO: 31 - protein, 713 aa, Campylobacter jejuni strain ATCC 700819 / NCTC 11168; identical to SEQ ID NO: 5

SEQ ID NO: 32 - protein, 416 aa, Artificial Sequence
  transmembrane domaine deleted alpha-1,3-mannosyl-glycoprotein 2-beta-N-acetylglucosaminyltransferase
TRPAPGRPPSVSALDGDPASLTREVIRLAQDAEVELERQRGLLQQIGDALSSQRGRVPTAAPPAQPRVPVTPAPAVIPILVIACDRSTVRRCLDKLLHYRPSAELFPIIVSQDCGHEETAQAIASYGSAVTHIRQPDLSSIAVPPDHRKFQGYYKIARHYRWALGQVFRQFRFPAAVVVEDDLEVAPDFFEYFRATYPLLKADPSLWCVSAWNDNGKEQMVDASRPELLYRTDFFPGLGWLLLAELWAELEPKWPKAFWDDWMRRPEQRQGRACIRPEISRTMTFGRKGVSHGQFFDQHLKFIKLNQQFVHFTQLDLSYLQREAYDRDFLARVYGAPQLQVEKVRTNDRKELGEVRVQYTGRDSFKAFAKALGVMDDLKSGVPRAGYRGIVTFQFRGRRVHLAPPLTWEGYDPSWN

SEQ ID NO: 33 - protein, 418 aa, Artificial Sequence
  transmembrane domaine deleted alpha-1,6-mannosyl-glycoprotein 2-beta-N-acetylglucosaminyltransferase
RQRKNEALAPPLLDAEPARGAGGRGGDHPSVAVGIRRVSNVSAASLVPAVPQPEADNLTLRYRSLVYQLNFDQTLRNVDKAGTWAPRELVLVVQVHNRPEYLRLLLDSLRKAQGIDNVLVIFSHDFWSTEINQLIAGVNFCPVLQVFFPFSIQLYPNEFPGSDPRDCPRDLPKNAALKLGCINAEYPDSFGHYREAKFSQTKHHWWWKLHFVWERVKILRDYAGLILFLEEDHYLAPDFYHVFKKMWKLKQQECPECDVLSLGTYSASRSFYGMADKVDVKTWKSTEHNMGLALTRNAYQKLIECTDTFCTYDDYNWDWTLQYLTVSCLPKFWKVLVPQIPRIFHAGDCGMHHKKTCRPSTQSAQIESLLNNNKQYMFPETLTISEKFTVVAISPPRKNGGWGDIRDHELCKSYRRLQ

SEQ ID NO: 34 - protein, 354 aa, Artificial Sequence
  transmembrane domaine deleted beta-1,4-galactosyltransferase 1
RDLSRLPQLVGVSTPLQGGSNSAAAIGQSSGELRTGGARPPPPLGASSQPRPGGDSSPVVDSGPGPASNLTSVPVPHTTALSLPACPEESPLLVGPMLIEFNMPVDLELVAKQNPNVKMGGRYAPRDCVSPHKVAIIIPFRNRQEHLKYWLYYLHPVLQRQQLDYGIYVINQAGDTIFNRAKLLNVGFQEALKDYDYTCFVFSDVDLIPMNDHNAYRCFSQPRHISVAMDKFGFSLPYVQYFGGVSALSKQQFLTINGFPNNYWGWGGEDDDIFNRLVFRGMSISRPNAVVGRCRMIRHSRDKKNEPNPQRFDRIAHTKETMLSDGLNSLTYQVLDVQRYPLYTQITVDIGTPS

SEQ ID NO: 35 - protein, 416 aa, Artificial Sequence
  beta-1,4-mannosyltransferase
MKSTKKRIIIFVLGDVGHSPRICYHAISFSKLGWQVELCGYVEDTLPKIISSDPNITVHHMSNLKRKGGGTSVIFMVKKVLFQVLSIFKLLWELRGSDYILVQNPPSIPILPIAVLYKLTGCKLIIDWHNLAYSILQLKFKGNFYHPLVLISYMVEMIFSKFADYNLTVTEAMRKYLIQSFHLNPKRCAVLYDRPASQFQPLAGDISRQKALTTKAFIKNYIRDDFDTEKGDKIIVTSTSFTPDEDIGILLGALKIYENSYVKFDSSLPKILCFITGKGPLKEKYMKQVEEYDWKRCQIEFVWLSAEDYPKLLQLCDYGVSLHTSSSGLDLPMKILDMFGSGLPVIAMNYPVLDELVQHNVNGLKFVDRRELHESLIFAMKDADLYQKLKKNVTQEAENRWQSNWERTMRDLKLIH

SEQ ID NO: 36 - protein, 503 aa, Artificial Sequence
  alpha-1,3/1,6-mannosyltransferase
MIEKDKRTIAFIHPDLGIGGAERLVVDAALGLQQQGHSVIIYTSHCDKSHCFEEVKNGQLKVEVYGDFLPTNFLGRFFIVFATIRQLYLVIQLILQKKVNAYQLIIIDQLSTCIPLLHIFSSATLMFYCHFPDQLLAQRAGLLKKIYRLPFDLIEQFSVSAADTVVVNSNFTKNTFHQTFKYLSNDPDVIYPCVDLSTIEIEDIDKKFFKTVFNEGDRFYLSINRFEKKKDVALAIKAFALSEDQINDNVKLVICGGYDERVAENVEYLKELQSLADEYELSHTTIYYQEIKRVSDLESFKTNNSKIIFLTSISSSLKELLLERTEMLLYTPAYEHFGIVPLEAMKLGKPVLAVNNGGPLETIKSYVAGENESSATGWLKPAVPIQWATAIDESRKILQNGSVNFERNGPLRVKKYFSREAMTQSFEENVEKVIWKEKKYYPWEIFGISFSNFILHMAFIKILPNNPWPFLFMATFMVLYFKNYLWGIYWAFVFALSYPYEEI

SEQ ID NO: 37 - protein, 826 aa, Artificial Sequence
  STT3A oligosaccharyltransferase from T. brucei
TKGGKVAVTKGSAQSDGAGEGGMSKAKSSTTFVATGGGSLPAWALKAVSTIVSAVILIYSVHRAYDIRLTSVRLYGELIHEFDPWFNYRATQYLSDNGWRAFFQWYDYMSWYPLGRPVGTTIFPGMQLTGVAIHRVLEMLGRGMSFPGMQLTGVAIHRVLEMLGRGMSINNICVYIPAWFGSIATVLAALIAYESSNSLSVMAFTAYFFSIVPAHLMRSMAGEFDNECVAMAAMLLTFYMWVRSLRSSSSWPIGALAGVAYGYMVSTWGYIFVLNMVAFHASVCVLLDWARGTYSVSLLRAYSLFFVIGTALAICVPPVEWTPFRSLEQLTALFVFVFMWALHYSEYLRERARAPIHSSKALQIRARIFMGTLSLLLIVASLLAPFGFFKPTAYRVRALFVKHTRTGNPLVDSVAEHRPTTAGAYLRYFHVCYPLWGCGGLSMLVFMKKDRWRAIVFLASLSTVTMYFSARMSRLLLLAGPAATACAGMFIGGLFDLALSQFGDLRSPKDASGDSDPAGGSKRAKGKVVNEPSERAIFSHRWFQRLVQSLPVPLRRGIAVVVLVCLFANPMRHSFEKSCEKMAHALSSPRIIAVTDLPNGERVLADDYYVSYLWLRNNTPEDARILSWWDYGYQITGIGNRTTLADGNTWSHKHIATIGKMLTSPVKESHALIRHLADYVLIWAGYDGSDLLKSPHMARIGNSVYRDMCSEDDPLCRQFGFYSGDLNKPTPMMQRSLLYNLHRFGTDGGKTQLDKNMFQLAYVSKYGLVKIYKVMNVSEESKAWVADPKNRVCDPPGSWICAGQYPPAKEIQDMLAKRFHYEASSR